European Patent Application EP 4 141 029 A1, published March 1, 2023. Title: ANTIBODY AGAINST NECTIN-4 AND APPLICATION THEREOF. Applicant: MABWELL (SHANGHAI) BIOSCIENCE CO., LTD. The sequence listing filed with the application follows.

SEQUENCE LISTING (97 sequences)

SEQ ID NO: 1 - protein, 447 aa, artificial sequence
  Enfortumab, HC
EVQLVESGGGLVQPGGSLRLSCAASGFTFSSYNMNWVRQAPGKGLEWVSYISSSSSTIYYADSVKGRFTISRDNAKNSLSLQMNSLRDEDTAVYYCARAYYYGMDVWGQGTTVTVSSASTKGPSVFPLAPSSKSTSGGTAALGCLVKDYFPEPVTVSWNSGALTSGVHTFPAVLQSSGLYSLSSVVTVPSSSLGTQTYICNVNHKPSNTKVDKRVEPKSCDKTHTCPPCPAPELLGGPSVFLFPPKPKDTLMISRTPEVTCVVVDVSHEDPEVKFNWYVDGVEVHNAKTKPREEQYNSTYRVVSVLTVLHQDWLNGKEYKCKVSNKALPAPIEKTISKAKGQPREPQVYTLPPSREEMTKNQVSLTCLVKGFYPSDIAVEWESNGQPENNYKTTPPVLDSDGSFFLYSKLTVDKSRWQQGNVFSCSVMHEALHNHYTQKSLSLSPGK

SEQ ID NO: 2 - protein, 214 aa, artificial sequence
  Enfortumab, LC
DIQMTQSPSSVSASVGDRVTITCRASQGISGWLAWYQQKPGKAPKFLIYAASTLQSGVPSRFSGSGSGTDFTLTISSLQPEDFATYYCQQANSFPPTFGGGTKVEIKRTVAAPSVFIFPPSDEQLKSGTASVVCLLNNFYPREAKVQWKVDNALQSGNSQESVTEQDSKDSTYSLSSTLTLSKADYEKHKVYACEVTHQGLSSPVTKSFNRGEC

SEQ ID NO: 3 - protein, 318 aa, Homo sapiens
GELETSDVVTVVLGQDAKLPCFYRGDSGEQVGQVAWARVDAGEGAQELALLHSKYGLHVSPAYEGRVEQPPPPRNPLDGSVLLRNAVQADEGEYECRVSTFPAGSFQARLRLRVLVPPLPSLNPGPALEEGQGLTLAASCTAEGSPAPSVTWDTEVKGTTSSRSFKHSRSAAVTSEFHLVPSRSMNGQPLTCVVSHPGLLQDQRITHILHVSFLAEASVRGLEDQNLWHIGREGAMLKCLSEGQPPPSYNWTRLDGPLPSGVRVDGDTLGFPPLTTEHSGIYVCHVSNEFSSRDSQVTVDVLDPQEDSGKQVDLVSAS

SEQ ID NO: 4 - protein, 330 aa, Homo sapiens
ASTKGPSVFPLAPSSKSTSGGTAALGCLVLDYFPEPVTVSWNSGALTSGVHTFPAVLQSSGLYSLSSVVTVPSSSLGTQTYICNVNHKPSNTKVDKRVEPKSCDKTHTCPPCPAPELLGGPSVFLFPPKPKDTLMISRTPEVTCVVVDVSHEDPEVLFNWYVDGVEVHNAKTKPREEQYNSTYRVVSVLTVLHQDWLNGKEYKCKVSNKALPAPIEKTISKAKGQPREPQVYTLPPSREEMTKNQVSLTCLVLGFYPSDIAVEWESNGQPENNYKTTPPVLDSDGSFFLYSKLTVDKSRWQQGNVFSCSVMHEALHNHYTQKSLSLSPGK

SEQ ID NO: 5 - protein, 107 aa, Homo sapiens [sequence omitted]

SEQ ID NO: 6 - protein, 510 aa, Cyno
MPLSLGAEMWGPEAWLLLLLLLASFTGRCPAGELETSDVVTVVLGQDAKLPCFYRGDSGEQVGQVAWARADAGEGAQELALLHSKYGLHVSPAYEGRVEQPPPPRNPLDGSVLLRNAVQADEGEYECRVSTFPAGSFQARLRLRVLVPPLPSLNPGPALEEGQGLTLAASCTAEGSPAPSVTWDTEVKGTTSSRSFKHSRSAAVTSEFHLVPSRSMNGQPLTCVVSHPGLLQDQRITHILHVSFLAEASVRGLEDQNLWHVGREGAMLKCLSEGQPPPSYNWTRLDGPLPSGVRVDGDTLGFPPLTTEHSGIYVCHVSNEFSSRDSQVTVDVLDPQEDSGKQVDLVSASVVVVGVIAALLFCLLVVVVVLMSRYHRRKAQQMTQKYEEELTLTRENSIRRLHSHHTDPRSQPEESVGLRAEGHPDSLKDNSSCSVMSEEPEGRSYSTLTTVREIETQTELLSPGSGRTEEEEDQDEGIKQAMNHFVQENGTLRAKPTGNGIYINGRGHLV

SEQ ID NO: 7 - protein, 116 aa, artificial sequence
  VH
QVQLQQSGPELVKPGASVRITCKASGYTFTTYYIHWVKQRPGQGLEWIGWIYPGNVNTKYNEKFKGKATLTADKSSSTAYMQLSSLTSEDSAVYFCARGLYYFDYWGQGTTLTVSS

SEQ ID NO: 8 - protein, 107 aa, artificial sequence
  VL
SIVMTQTPKFLLVSAGDRLTITCKASQSVSNDVAWYQQKPGQSPKLLIYYASNRYTGVPDRFTGSGYGTDFTFTISTVQAEDLAVYFCQQDYSSPYTFGGGTKLEIK

SEQ ID NO: 9 - protein, 116 aa, artificial sequence
  VH
QVQLVQSGAEVKKPGASVKVSCKASGYTFTTYYIHWVRQAPGQRLEWMGWIYPGNVNTKYNEKFKGRVTITRDTSASTAYMELSSLRSEDTAVYYCARGLYYFDYWGQGTLVTVSS

SEQ ID NO: 10 - protein, 116 aa, artificial sequence
  VH
QVQLVQSGAEVKKPGASVKVSCKASGYTFTTYYIHWVRQAPGQRLEWMGWIYPGNVNTKYNEKFKGRVTITADKSASTAYMELSSLRSEDTAVYYCARGLYYFDYWGQGTLVTVSS

SEQ ID NO: 11 - protein, 107 aa, artificial sequence
  VL
DIQMTQSPSSLSASVGDRVTITCKASQSVSNDVAWYQQKPGKVPKLLIYYASNRYTGVPSRFSGSGSGTDFTLTISSLQPEDVATYYCQQDYSSPYTFGGGTKVEIK

SEQ ID NO: 12 - protein, 107 aa, artificial sequence
  VL
DIQMTQSPSSLSASVGDRVTITCKASQSVSNDVAWYQQKPGKVPKLLIYYASNRYTGVPSRFSGSGSGTDFTLTISSLQPEDLATYFCQQDYSSPYTFGGGTKVEIK

SEQ ID NO: 13 - protein, 119 aa, artificial sequence
  VH
QVQLKESGPGLVAPSQSLSISCTVSGFSLIDYGVSWIRQPPGKGLEWLGVIWGDGKIYYNSVLKSRLSISKDNSKSQVFLKMNSLQTDDTAMYYCAKQGGLLFYAMDYWGQGTSVTVSS

SEQ ID NO: 14 - protein, 113 aa, artificial sequence
  VL
DIVMTQSPSSLAMSVGQRVTMNCKSSQSLLNSYSQKNYLAWYQQKPGQSPKLLIYFASTRESGVPDRFIGSGSETDFTLTISSVQAEDLADYFCQQHYNTPFTFGSGTKLEIK

SEQ ID NO: 15 - protein, 119 aa, artificial sequence
  VH
QVQLQESGPGLVKPSETLSLTCTVSGFSLIDYGVSWIRQPPGKGLEWIGVIWGDGKIYYNSVLKSRVTISVDTSKNQFSLKLSSVTAADTAVYYCARQGGLLFYAMDYWGQGTLVTVSS

SEQ ID NO: 16 - protein, 119 aa, artificial sequence
  VH
QVQLQESGPGLVKPSETLSLTCTVSGFSLIDYGVSWIRQPPGKGLEWIGVIWGDGKIYYNSVLKSRVTISKDNSKSQVSLKLSSVTAADTAVYYCAKQGGLLFYAMDYWGQGTLVTVSS

SEQ ID NO: 17 - protein, 119 aa, artificial sequence
  VH
QVQLQESGPGLVKPSETLSLTCTVSGFSLIDYGVSWIRQPPGKGLEWIGVIWGEGKIYYNSVLKSRVTISKDNSKSQVSLKLSSVTAADTAVYYCAKQGGLLFYAMDYWGQGTLVTVSS

SEQ ID NO: 18 - protein, 119 aa, artificial sequence
  VH
QVQLQESGPGLVKPSETLSLTCTVSGFSLIDYGVSWIRQPPGKGLEWIGVIWGDGKIYYNSVLKSRVTISKDNSKSQVSLKLSSVTAADTAVYYCARQGGLLFYAMDYWGQGTLVTVSS

SEQ ID NO: 19 - protein, 119 aa, artificial sequence
  VH
QVQLQESGPGLVKPSETLSLTCTVSGFSLIDYGVSWIRQPPGKGLEWIGVIWGDAKIYYNSVLKSRVTISKDNSKSQVSLKLSSVTAADTAVYYCAKQGGLLFYAMDYWGQGTLVTVSS

SEQ ID NO: 20 - protein, 119 aa, artificial sequence
  VH
QVQLQESGPGLVKPSETLSLTCTVSGFSLIDYGVSWIRQPPGKGLEWIGVIWGGDKIYYNSVLKSRVTISKDNSKSQVSLKLSSVTAADTAVYYCAKQGGLLFYAMDYWGQGTLVTVSS

SEQ ID NO: 21 - protein, 119 aa, artificial sequence
  VH
QVQLQESGPGLVKPSETLSLTCTVSGFSLIDYGVSWIRQPPGKGLEWIGVIWGGGKIYYNSVLKSRVTISKDNSKSQVSLKLSSVTAADTAVYYCAKQGGLLFYAMDYWGQGTLVTVSS

SEQ ID NO: 22 - protein, 114 aa, artificial sequence
  VL
DIVMTQSPDSLAVSLGERATINCKSSQSLLNSYSQKNYLAWYQQKPGQPPKLLIYFASTRESGVPDRFSGSGSGTDFTLTISSLQAEDVAVYYCQQHYNTPFTFGAGTKLELKR

SEQ ID NO: 23 - protein, 114 aa, artificial sequence
  VL
DIVMTQSPDSLAVSLGERATINCKSSQSLLNSYSQKNYLAWYQQKPGQSPKLLIYFASTRESGVPDRFSGSGSETDFTLTISSLQAEDLAVYFCQQHYNTPFTFGAGTKLELKR

SEQ ID NO: 24 - protein, 114 aa, artificial sequence
  VL
DIVMTQSPDSLAVSLGERATINCKSSQSLLYSYSQKNYLAWYQQKPGQSPKLLIYFASTRESGVPDRFSGSGSETDFTLTISSLQAEDLAVYFCQQHYNTPFTFGAGTKLELKR

SEQ ID NO: 25 - protein, 114 aa, artificial sequence
  VL
DIVMTQSPDSLAVSLGERATINCKSSQSLLNTYSQKNYLAWYQQKPGQSPKLLIYFASTRESGVPDRFSGSGSETDFTLTISSLQAEDLAVYFCQQHYNTPFTFGAGTKLELKR

SEQ ID NO: 26 - protein, 114 aa, artificial sequence
  VL
DIVMTQSPDSLAVSLGERATINCKSSQSLLNKYSQKNYLAWYQQKPGQPPKLLIYFASTRESGVPDRFSGSGSGTDFTLTISSLQAEDVAVYYCQQHYNTPFTFGAGTKLELKR

SEQ ID NO: 27 - protein, 116 aa, artificial sequence
  VH
QVQLQQSGPELVKPGASVRISCKASGYTFTSYYIHWVKQRPGQGLEWIGWIYPGNANNKYNENFKGKATLTADKSSSTAYMQLSSLTSEDSAVYFCARSVYYFDYWGQGTTLTVSS

SEQ ID NO: 28 - protein, 107 aa, artificial sequence
  VL
SVVMTQTPKFLLVSAGDRVTITCKASQSVSNDVAWYQQKPGQSPKLLIYYASNRNTGVPDRFTGSGYGTDFTFNISTVQAEDLAVYFCQQDYSSPYTFGGGTKLEIK

SEQ ID NO: 29 - protein, 116 aa, artificial sequence
  VH
QVQLVQSGAEVKKPGASVKVSCKASGYTFTSYYIHWVRQAPGQRLEWMGWIYPGNANNKYNENFKGRVTITRDTSASTAYMELSSLRSEDTAVYYCARSVYYFDYWGQGTLVTVSS

SEQ ID NO: 30 - protein, 116 aa, artificial sequence
  VH
QVQLVQSGAEVKKPGASVKVSCKASGYTFTSYYIHWVRQAPGQRLEWMGWIYPGNANNKYNENFKGRVTITADKSASTAYMELSSLRSEDTAVYYCARSVYYFDYWGQGTLVTVSS

SEQ ID NO: 31 - protein, 107 aa, artificial sequence
  VL
EIVMTQSPATLSVSPGERATLSCKASQSVSNDVAWYQQKPGQAPRLLIYYASNRNTGIPARFSGSGSGTEFTLTISSLQSEDFAVYYCQQDYSSPYTFGGGTKVEIK

SEQ ID NO: 32 - protein, 107 aa, artificial sequence
  VL
EVVMTQSPATLSVSPGERATLSCKASQSVSNDVAWYQQKPGQAPRLLIYYASNRNTGIPARFSGSGSGTEFTLTISSLQSEDLAVYFCQQDYSSPYTFGGGTKVEIK

SEQ ID NO: 33 - protein, 117 aa, artificial sequence
  VH
EVQLQQSGPDLVKPGASVKISCKASGYSFTDYYMHWVKQSRGKGLEWIGRVNPNNGNTLYNQKFRGKAILTVDKSSSTAYMELRSLTSDDSAVYYCAREDRYAFAYWGQGTLVTVSA

SEQ ID NO: 34 - protein, 111 aa, artificial sequence
  VL
DIVLTQSPASLAVSLGQRATISCRASQSVSTSSYTYMHWYQQKPGQPPKLLIKYASNLESGVPARFIGSGSGTDFTLNIHPVEEEDTATYYCQHTWEIPYTFGGGTKLEIK

SEQ ID NO: 35 - protein, 7 aa, artificial sequence
  CDR-H1
GYTFTTY

SEQ ID NO: 36 - protein, 10 aa, artificial sequence
  CDR-H1
GYTFTTYYIH

SEQ ID NO: 37 - protein, 5 aa, artificial sequence
  CDR-H1
TYYIH

SEQ ID NO: 38 - protein, 6 aa, artificial sequence
  CDR-H1
TTYYIH

SEQ ID NO: 39 - protein, 6 aa, artificial sequence
  CDR-H2
YPGNVN

SEQ ID NO: 40 - protein, 10 aa, artificial sequence
  CDR-H2
WIYPGNVNTK

SEQ ID NO: 41 - protein, 17 aa, artificial sequence
  CDR-H2
WIYPGNVNTKYNEKFKG

SEQ ID NO: 42 - protein, 13 aa, artificial sequence
  CDR-H2
WIGWIYPGNVNTK

SEQ ID NO: 43 - protein, 7 aa, artificial sequence
  CDR-H3
GLYYFDY

SEQ ID NO: 44 - protein, 8 aa, artificial sequence
  CDR-H3
ARGLYYFD

SEQ ID NO: 45 - protein, 11 aa, artificial sequence
  CDR-L1
KASQSVSNDVA

SEQ ID NO: 46 - protein, 7 aa, artificial sequence
  CDR-L1
SNDVAWY

SEQ ID NO: 47 - protein, 7 aa, artificial sequence
  CDR-L2
YASNRYT

SEQ ID NO: 48 - protein, 10 aa, artificial sequence
  CDR-L2
LLIYYASNRY

SEQ ID NO: 49 - protein, 9 aa, artificial sequence
  CDR-L3
QQDYSSPYT

SEQ ID NO: 50 - protein, 8 aa, artificial sequence
  CDR-L3
QQDYSSPY

SEQ ID NO: 51 - protein, 7 aa, artificial sequence
  CDR-H1
GFSLIDY

SEQ ID NO: 52 - protein, 10 aa, artificial sequence
  CDR-H1
GFSLIDYGVS

SEQ ID NO: 53 - protein, 5 aa, artificial sequence
  CDR-H1
DYGVS

SEQ ID NO: 54 - protein, 6 aa, artificial sequence
  CDR-H1
IDYGVS

SEQ ID NO: 55 - protein, 5 aa, artificial sequence
  CDR-H2
WGDGK

SEQ ID NO: 56 - protein, 9 aa, artificial sequence
  CDR-H2
VIWGDGKIY

SEQ ID NO: 57 - protein, 16 aa, artificial sequence
  CDR-H2
VIWGDGKIYYNSVLKS

SEQ ID NO: 58 - protein, 12 aa, artificial sequence
  CDR-H2
WLGVIWGDGKIY

SEQ ID NO: 59 - protein, 11 aa, artificial sequence
  CDR-H3
QGGLLFYAMDY

SEQ ID NO: 60 - protein, 12 aa, artificial sequence
  CDR-H3
AKQGGLLFYAMD

SEQ ID NO: 61 - protein, 17 aa, artificial sequence
  CDR-L1
KSSQSLLNSYSQKNYLA

SEQ ID NO: 62 - protein, 13 aa, artificial sequence
  CDR-L1
LNSYSQKNYLAWY

SEQ ID NO: 63 - protein, 7 aa, artificial sequence
  CDR-L2
FASTRES

SEQ ID NO: 64 - protein, 10 aa, artificial sequence
  CDR-L2
LLIYFASTRE

SEQ ID NO: 65 - protein, 9 aa, artificial sequence
  CDR-L3
QQHYNTPFT

SEQ ID NO: 66 - protein, 8 aa, artificial sequence
  CDR-L3
QQHYNTPF

SEQ ID NO: 67 - protein, 17 aa, artificial sequence
  CDR-L1
KSSQSLLNTYSQKNYLA

SEQ ID NO: 68 - protein, 5 aa, artificial sequence
  CDR-H2
WGDAK

SEQ ID NO: 69 - protein, 5 aa, artificial sequence
  CDR-H2
WGGGK

SEQ ID NO: 70 - protein, 7 aa, artificial sequence
  CDR-H1
GYTFTSY

SEQ ID NO: 71 - protein, 10 aa, artificial sequence
  CDR-H1
GYTFTSYYIH

SEQ ID NO: 72 - protein, 5 aa, artificial sequence
  CDR-H1
SYYIH

SEQ ID NO: 73 - protein, 6 aa, artificial sequence
  CDR-H1
TSYYIH

SEQ ID NO: 74 - protein, 6 aa, artificial sequence
  CDR-H2
YPGNAN

SEQ ID NO: 75 - protein, 10 aa, artificial sequence
  CDR-H2
WIYPGNANNK

SEQ ID NO: 76 - protein, 17 aa, artificial sequence
  CDR-H2
WIYPGNANNKYNENFKG

SEQ ID NO: 77 - protein, 13 aa, artificial sequence
  CDR-H2
WIGWIYPGNANNK

SEQ ID NO: 78 - protein, 7 aa, artificial sequence
  CDR-H3
SVYYFDY

SEQ ID NO: 79 - protein, 8 aa, artificial sequence
  CDR-H3
ARSVYYFD

SEQ ID NO: 80 - protein, 7 aa, artificial sequence
  CDR-L2
YASNRNT

SEQ ID NO: 81 - protein, 10 aa, artificial sequence
  CDR-L2
LLIYYASNRN

SEQ ID NO: 82 - protein, 7 aa, artificial sequence
  CDR-H1
GYSFTDY

SEQ ID NO: 83 - protein, 10 aa, artificial sequence
  CDR-H1
GYSFTDYYMH

SEQ ID NO: 84 - protein, 5 aa, artificial sequence
  CDR-H1
DYYMH

SEQ ID NO: 85 - protein, 6 aa, artificial sequence
  CDR-H1
TDYYMH

SEQ ID NO: 86 - protein, 6 aa, artificial sequence
  CDR-H2
NPNNGN

SEQ ID NO: 87 - protein, 10 aa, artificial sequence
  CDR-H2
RVNPNNGNTL

SEQ ID NO: 88 - protein, 17 aa, artificial sequence
  CDR-H2
RVNPNNGNTLYNQKFRG

SEQ ID NO: 89 - protein, 13 aa, artificial sequence
  CDR-H2
WIGRVNPNNGNTL

SEQ ID NO: 90 - protein, 8 aa, artificial sequence
  CDR-H3
EDRYAFAY

SEQ ID NO: 91 - protein, 9 aa, artificial sequence
  CDR-H3
AREDRYAFA

SEQ ID NO: 92 - protein, 15 aa, artificial sequence
  CDR-L1
RASQSVSTSSYTYMH

SEQ ID NO: 93 - protein, 11 aa, artificial sequence
  CDR-L1
STSSYTYMHWY

SEQ ID NO: 94 - protein, 7 aa, artificial sequence
  CDR-L2
YASNLES

SEQ ID NO: 95 - protein, 10 aa, artificial sequence
  CDR-L2
LLIKYASNLE

SEQ ID NO: 96 - protein, 9 aa, artificial sequence
  CDR-L3
QHTWEIPYT

SEQ ID NO: 97 - protein, 8 aa, artificial sequence
  CDR-L3
QHTWEIPY